European Patent Application EP 4 239 071 A1, published September 6, 2023. Title: Protease mutant and use thereof. Applicant: Kao Corporation. The sequence listing filed with the application follows.

SEQUENCE LISTING (2 sequences)

SEQ ID NO: 1 - DNA, 1134 bp, Achromobacter lyticus
atgaaaaaaatctcaaaagctggtctgggactggctctggtctgtgctctggcgacgattggaggcaacgcatctgctcagggacatggattaagcggcgaagatctggtttactcttacgatgaaatgtttgattttgatatcgatgcctacctggcaaaacatgcgccgcatctgcataaacatagcgaagaaatctctcattgggccggatattctggcatttcaccgaaagttcttatcgcattaatggaacaacagtcaggagctgtgagcgccaaaagagcaacaaatcgcccgtttggcaaacttgccagagcagatggatttggcgcccaaacacgcgaagtggcgttagctctgagagaatctctttatgaacgcgatccggatggagccaaaggcccggtcacattagccagagcaaacccgctgcaggcactttttgaacgctcaggagataatgaaccggcagcggctttaagaggagatggcgaatttcaacttgtctacggcagattatttaacgaaccgcgccaggcaaaagccgcaagcgatagatttgcgaaagctggaccggatgttcaaccgttatctccgaatggactgcttcagtttccgtttccgagaggcgcatcttggcatgtgggcggagctcatacaaacacaggatcaggcaattatccgatgtcaagcctggatatgtcaagaggcggaggctggggaagcaatcaaaacggcaattgggtttcagcgagcgcggctggatcttttaaacgccattcttcatgctttgctgaaattgttcatacaggcggctggtcaacaacatactaccatctgatgaacatccagtacaatacaggcgcgaacgttagcatgaatacagccatcgcaaacccggctaatacacaagcgcaggctctgtgcaacggaggccaaagcacaggaccgcatgaacattggtcactgaaacagaacggctcattttaccatctgaacggaacatacctttcaggctatagaatcacagcgacaggcagctcttatgatacaaattgtagccgcttttatttgacaaaaaatggacagaactactgctatggttattatgtgaatcctggaccgaactaa

SEQ ID NO: 2 - protein, 179 aa, Achromobacter lyticus
  beta-lytic metallopeptidase (BLP) mature protein
SPNGLLQFPFPRGASWHVGGAHTNTGSGNYPMSSLDMSRGGGWGSNQNGNWVSASAAGSFKRHSSCFAEIVHTGGWSTTYYHLMNIQYNTGANVSMNTAIANPANTQAQALCNGGQSTGPHEHWSLKQNGSFYHLNGTYLSGYRITATGSSYDTNCSRFYLTKNGQNYCYGYYVNPGPN